European Patent Application EP 4 538 705 A2, published April 16, 2025. Title: IMMUNOASSAY TEST DEVICE WITH TWO FLUID FLOW PATHS FOR DETECTION AND DIFFERENTIATION OF TWO OR MORE ANALYTES. Applicant: QUIDEL CORPORATION. The sequence listing filed with the application follows.

SEQUENCE LISTING (21 sequences)

SEQ ID NO: 1 - protein, 17 aa, Borrelia burgdorferi
MKKNDQIVAAIALRGVA

SEQ ID NO: 2 - protein, 26 aa, Borrelia burgdorferi
CMKKDDQIAAAMVLRGMAKDGQFALK

SEQ ID NO: 3 - protein, 17 aa, Borrelia burgdorferi
MKKNDQIGAAIALRGVA

SEQ ID NO: 4 - protein, 17 aa, Borrelia burgdorferi
MKKDDQIAAAIALRGMA

SEQ ID NO: 5 - protein, 26 aa, Borrelia burgdorferi
MKKDDQIAAAMVLRGMAKDGQFALKD

SEQ ID NO: 6 - protein, 26 aa, Borrelia burgdorferi
MKKDDQIAAAIALRGMAKDGKFAVKD

SEQ ID NO: 7 - protein, 13 aa, Borrelia burgdorferi
VQEGVQQEGAQQP

SEQ ID NO: 8 - protein, 10 aa, Borrelia burgdorferi
PVVAESPKKP

SEQ ID NO: 9 - protein, 11 aa, Borrelia burgdorferi
CPVVAESPKKP

SEQ ID NO: 10 - protein, 12 aa, Borrelia burgdorferi
LCPVVAESPKKP

SEQ ID NO: 11 - protein, 35 aa, Borrelia burgdorferi
YGQNWTNPENMVTSGPFKLKERIPNEKIVFEKNNK

SEQ ID NO: 12 - protein, 20 aa, Borrelia burgdorferi
MTLFLFISCNNSGKDGNTSA

SEQ ID NO: 13 - protein, 21 aa, Borrelia burgdorferi
KMTLFLFISCNNSGKDGNTSA

SEQ ID NO: 14 - protein, 15 aa, Borrelia burgdorferi
TILVNLLISCGLTGA

SEQ ID NO: 15 - protein, 30 aa, Borrelia burgdorferi
KDLKNKILKIKKEATGKGVLFEAFTGLKTG

SEQ ID NO: 16 - protein, 56 aa, synthetic construct
  REGION 1..56: note = Synthetic
VQEGVQQEGAQQPGGGMTLFLFISCNNSGKDGNTSAGGGMKKNDQIVAAIALRGVA

SEQ ID NO: 17 - protein, 33 aa, synthetic construct
  REGION 1..33: note = Synthetic
VQEGVQQEGAQQPGGGMKKNDQIVAAIALRGVA

SEQ ID NO: 18 - protein, 42 aa, synthetic construct
  REGION 1..42: note = Synthetic
VQEGVQQEGAQQPGGGMKKDDQIAAAMVLRGMAKDGQFALKD

SEQ ID NO: 19 - protein, 4 aa, synthetic construct
  REGION 1..4: note = Synthetic
GGGG

SEQ ID NO: 20 - protein, 212 aa, Borrelia burgdorferi
MKKNTLSAILMTLFLFISCNNSGKDGNTSANSADESVKGPNLTEISKKITESNAVVLAVKEVETLLASIDEVAKKAIGNLIAQNGLNAGANQNGSLLAGAYVISTLIAEKLDGLKNSEELKEKIEDAKKCNKAFTDKLKSSHAELGIANGAATDANAKAAILKTNGTKDKGAQELEKLFESVKNLSKAAQETLNNSVKELTSPVVAENPKKP

SEQ ID NO: 21 - protein, 191 aa, Borrelia burgdorferi
MIKCNNKTFNNLLKLTILVNLLISCGLTGATKIRLERSAKDITDEIDAIKKDAALKGVNFDAFKDKKTGSGVSENPFILEAKVRATTVAEKFVIAIEEEATKLKETGSSGEFSAMYDLMFEVSKPLQKLGIQEMTKTVSDAAEENPPTTAQGVLEIAKKMREKLQRVHTKNYCTLKKKENSTFTDEKCKNN